European Patent Specification EP 3 579 875 B1, published January 22, 2025. Title: Specific Binding Molecules. Applicant: Medannex Ltd. The sequence listing filed with the application follows.

SEQUENCE LISTING (92 sequences)

SEQ ID NO: 1 - protein, 16 aa, Mus musculus
RSSQSLENSNGKTYLN

SEQ ID NO: 2 - protein, 7 aa, Mus musculus
GVSNRFS

SEQ ID NO: 3 - protein, 9 aa, Mus musculus
LQVTHVPYT

SEQ ID NO: 4 - protein, 10 aa, Mus musculus
GYTFTNYWIG

SEQ ID NO: 5 - protein, 17 aa, Mus musculus
DIYPGGDYTNYNEKFKG

SEQ ID NO: 6 - protein, 11 aa, Mus musculus
ARWGLGYYFDY

SEQ ID NO: 7 - protein, 11 aa, Mus musculus
KASENVVTYVS

SEQ ID NO: 8 - protein, 7 aa, Mus musculus
GASNRYT

SEQ ID NO: 9 - protein, 9 aa, Mus musculus
GQGYSYPYT

SEQ ID NO: 10 - protein, 346 aa, Homo sapiens
MAMVSEFLKQAWFIENEEQEYVQTVKSSKGGPGSAVSPYPTFNPSSDVAALHKAIMVKGVDEATIIDILTKRNNAQRQQIKAAYLQETGKPLDETLKKALTGHLEEVVLALLKTPAQFDADELRAAMKGLGTDEDTLIEILASRTNKEIRDINRVYREELKRDLAKDITSDTSGDFRNALLSLAKGDRSEDFGVNEDLADSDARALYEAGERRKGTDVNVFNTILTTRSYPQLRRVFQKYTKYSKHDMNKVLDLELKGDIEKCLTAIVKCATSKPAFFAEKLHQAMKGVGTRHKALIRIMVSRSEIDMNDIKAFYQKMYGISLCQAILDETKGDYEKILVALCGGN

SEQ ID NO: 11 - protein, 346 aa, Homo sapiens; identical to SEQ ID NO: 10

SEQ ID NO: 12 - protein, 204 aa, Homo sapiens
MNLILRYTFSKMAMVSEFLKQAWFIENEEQEYVQTVKSSKGGPGSAVSPYPTFNPSSDVAALHKAIMVKGVDEATIIDILTKRNNAQRQQIKAAYLQETGKPLDETLKKALTGHLEEVVLALLKTPAQFDADELRAAMKGLGTDEDTLIEILASRTNKEIRDINRVYREELKRDLAKDITSDTSGDFRNALLSLAKGDRSEDFG

SEQ ID NO: 13 - protein, 115 aa, Homo sapiens
MAMVSEFLKQAWFIENEEQEYVQTVKSSKGGPGSAVSPYPTFNPSSDVAALHKAIMVKGVDEATIIDILTKRNNAQRQQIKAAYLQETGKPLDETLKKALTGHLEEVVLALLKTP

SEQ ID NO: 14 - protein, 9 aa, Mus musculus
WGLGYYFDY

SEQ ID NO: 15 - protein, 239 aa, Mus musculus
MVSSAQFLGLLLLCFQGTRCDAVMTQTPLSLPVSLGDQVSISCRSSQSLENSNGKTYLNWYLQKPGQSPQLLIYGVSNRFSGVLDRFSGSGSGTDFTLKISRVEAEDLGVYFCLQVTHVPYTFGGGTKLEIKRADAAPTVSIFPPSSEQLTSGGASVVCFLNNFYPKDINVKWKIDGSERQNGVLNSWTDQDSKDSTYSMSSTLTLTKDEYERHNSYTCEATHKTSTSPIVKSFNRNEC

SEQ ID NO: 16 - protein, 473 aa, Mus musculus
MGWTLVFLFLLSVTAGVHSQVQLQQSGPELVRPGTSVKMSCKASGYTFTNYWIGWAKQRPGHGLEWIGDIYPGGDYTNYNEKFKGKATLTADKSSSTAYMQFSSLTSEDSAIYYCARWGLGYYFDYWGQGITLTVSSAKTTPPSVYPLAPGCGDTTGSSVTLGCLVKGYFPESVTVTWNSGSLSSSVHTFPALLQSGLYTMSSSVTVPSSTWPSQTVTCSVAHPASSTTVDKKLEPSGPISTINPCPPCKECHKCPAPNLEGGPSVFIFPPNIKDVLMISLTPKVTCVVVDVSEDDPDVQISWFVNNVEVHTAQTQTHREDYNSTIRVVSTLPIQHQDWMSGKEFKCKVNNKDLPSPIERTISKIKGLVRAPQVYILPPPAEQLSRKDVSLTCLVVGFNPGDISVEWTSNGHTEENYKDTAPVLDSDGSYFIYSKLNMKTSKWEKTDSFSCNVRHEGLKNYYLKKTISRSPGK

SEQ ID NO: 17 - protein, 70 aa, Artificial Sequence
  Combined sequence of Mdx001 CDRs
RSSQSLENSNGKTYLNGVSNRFSLQVTHVPYTGYTFTNYWIGDIYPGGDYTNYNEKFKGARWGLGYYFDY

SEQ ID NO: 18 - protein, 112 aa, Mus musculus
DAVMTQTPLSLPVSLGDQVSISCRSSQSLENSNGKTYLNWYLQKPGQSPQLLIYGVSNRFSGVLDRFSGSGSGTDFTLKISRVEAEDLGVYFCLQVTHVPYTFGGGTKLEIK

SEQ ID NO: 19 - protein, 118 aa, Mus musculus
QVQLQQSGPELVRPGTSVKMSCKASGYTFTNYWIGWAKQRPGHGLEWIGDIYPGGDYTNYNEKFKGKATLTADKSSSTAYMQFSSLTSEDSAIYYCARWGLGYYFDYWGQGITLTVSS

SEQ ID NO: 20 - DNA, 48 bp, Artificial Sequence
  Mdx001 VLCDR1 Sequence Codon-Optimised for Expression in Hamster
cggtcaagccagagcttggagaactcgaatggaaagacctacctcaat

SEQ ID NO: 21 - DNA, 21 bp, Artificial Sequence
  Mdx001 VLCDR2 Sequence Codon-Optimised for Expression in Hamster
ggggtgtcgaacagattttcc

SEQ ID NO: 22 - DNA, 27 bp, Artificial Sequence
  Mdx001 VLCDR3 Sequence Codon-Optimised for Expression in Hamster
cttcaggtcacccatgtgccgtacacc

SEQ ID NO: 23 - DNA, 30 bp, Artificial Sequence
  Mdx001 VHCDR1 Sequence Codon-Optimised for Expression in Hamster
ggctacaccttcaccaactactggatcggc

SEQ ID NO: 24 - DNA, 51 bp, Artificial Sequence
  Mdx001 VLCDR2 Sequence Codon-Optimised for Expression in Hamster
gacatctatccgggtggagactacaccaactacaacgaaaagttcaaggga

SEQ ID NO: 25 - DNA, 33 bp, Artificial Sequence
  Mdx001 VHCDR3 Sequence Codon-Optimised for Expression in Hamster
gcccggtggggacttggttactacttcgactac

SEQ ID NO: 26 - DNA, 321 bp, Mus musculus
cagactccactctccctgcctgtcagtcttggagatcaagtctccatctcttgcaggtctagtcagagccttgaaaacagtaatggaaaaacctatttgaactggtacctccagaaaccaggccagtctccacagctcctgatctacggggtttccaaccgattttctggggtcctagacaggttcagtggtagtggatcagggacagatttcacactgaaaatcagcagagtggaggctgaggatttgggagtttatttctgcctccaagttacacatgtcccgtacacgttcggaggggggaccaagctggaaataaaa

SEQ ID NO: 27 - DNA, 357 bp, Mus musculus
ccaggtccagctgcagcagtctggacctgaactggtcaggcctgggacttcagtgaagatgtcctgcaaggcttctggatacaccttcactaactactggataggttgggcaaagcagaggcctggacatggccttgagtggattggagatatttaccctggaggtgattatactaactacaatgagaagttcaagggcaaggccacactgactgcagacaaatcctccagcacagcctacatgcagttcagcagcctgacatctgaggactctgccatctattattgtgcaagatgggggttaggatactactttgactactggggccaaggcatcactctcacagtctcctcagc

SEQ ID NO: 28 - DNA, 336 bp, Artificial Sequence
  Mdx001 Light Chain Variable Region Codon-Optimised for Expression in Hamster
gacgctgtgatgacccagactcctctgtccctgcccgtgtccctgggggaccaagtctccatctcctgccggtcaagccagagcttggagaactcgaatggaaagacctacctcaattggtacctccagaagccggggcagtccccccaactcctgatctacggggtgtcgaacagattttccggagtgctggatcggttctcgggctccggaagcggcaccgacttcactctgaaaattagccgcgtggaagccgaggacttgggcgtgtatttctgccttcaggtcacccatgtgccgtacaccttcggtggcggcacaaagctggaaatcaag

SEQ ID NO: 29 - DNA, 354 bp, Artificial Sequence
  Mdx001 Heavy Chain Variable Region Codon-Optimised for Expression in Hamster
caagtgcagctgcagcagtccggccccgaactcgtgcggccaggcacctccgtgaagatgtcctgcaaagcgtccggctacaccttcaccaactactggatcggctgggcaaagcagaggcccggacatggcctcgaatggattggcgacatctatccgggtggagactacaccaactacaacgaaaagttcaagggaaaggccaccctgaccgctgataagtccagctccaccgcatacatgcagttctcgtcactgactagcgaagattccgcgatctactactgcgcccggtggggacttggttactacttcgactactggggacagggaattaccctgaccgtgtccagc

SEQ ID NO: 30 - DNA, 717 bp, Artificial Sequence
  Mdx001 Light Chain Codon-Optimised for Expression in Hamster
atggtgtcatctgcacaatttctgggacttcttctgctgtgtttccaaggaacccgctgtgacgctgtgatgacccagactcctctgtccctgcccgtgtccctgggggaccaagtctccatctcctgccggtcaagccagagcttggagaactcgaatggaaagacctacctcaattggtacctccagaagccggggcagtccccccaactcctgatctacggggtgtcgaacagattttccggagtgctggatcggttctcgggctccggaagcggcaccgacttcactctgaaaattagccgcgtggaagccgaggacttgggcgtgtatttctgccttcaggtcacccatgtgccgtacaccttcggtggcggcacaaagctggaaatcaagagggcggacgcggcccctaccgtgtcaattttcccaccgagctccgaacagctcaccagcggcggtgcctcggtcgtgtgcttcctcaacaacttctatccaaaagacattaacgtcaagtggaagatcgatggatcggagagacagaacggagtgctgaacagctggactgatcaggactccaaggattcgacctactccatgagctccactctgaccctgaccaaggacgaatacgagcggcacaattcctacacttgcgaagccacccacaagacctcaacgtcccccatcgtgaagtccttcaaccgcaacgagtgc

SEQ ID NO: 31 - DNA, 1422 bp, Artificial Sequence
  Mdx001 Heavy Chain Codon-Optimised for Expression in Hamster
atgggatggactctcgtgttcctttttctcctctctgtcactgccggggtgcattcgcaagtgcagctgcagcagtccggccccgaactcgtgcggccaggcacctccgtgaagatgtcctgcaaagcgtccggctacaccttcaccaactactggatcggctgggcaaagcagaggcccggacatggcctcgaatggattggcgacatctatccgggtggagactacaccaactacaacgaaaagttcaagggaaaggccaccctgaccgctgataagtccagctccaccgcatacatgcagttctcgtcactgactagcgaagattccgcgatctactactgcgcccggtggggacttggttactacttcgactactggggacagggaattaccctgaccgtgtccagcgccaagactacgccgccgtccgtctaccctttggcccccggttgcggcgacaccaccggctcgtcagtgactctgggctgcctcgtgaaggggtacttccccgagtccgtcaccgtcacttggaacagcggcagcctttcgtcctcggtccacaccttccccgctctgctgcaaagcggtctgtacaccatgtcctcatccgtgaccgtgccctcctccacttggccgagccagaccgtgacttgctccgtggcccacccggcgtcctcgaccaccgtggacaagaagctggagccgtcaggtccaatctccaccatcaatccctgcccgccttgtaaagagtgccacaagtgccctgcccccaatctggagggaggaccttcggtgttcattttccctccgaatatcaaggacgtgttgatgatctccctgaccccgaaggtcacatgcgtggtcgtcgacgtgtccgaggacgatccggacgtgcagattagctggttcgtgaacaacgtggaagtgcacactgcgcagacccaaacccatcgggaggactataactccactatccgcgtcgtgtcaacactgccgatccagcaccaggactggatgagcggaaaggaattcaagtgtaaagtcaacaacaaggatctgccaagccctatcgagcgcaccattagcaagatcaagggactcgtgcgcgccccacaagtgtacattctcccccctccggcggaacagctgagcagaaaggatgtgtcgctgacgtgtttggtcgtgggattcaaccccggggatatttccgtggaatggacttcgaacgggcacaccgaagagaactacaaggacaccgcccctgtgctggacagcgacggatcatacttcatctattcgaagctgaacatgaaaacttccaaatgggaaaagaccgactcgttttcctgtaacgtgcgccacgaaggactcaagaactactacctgaagaaaactatctctcggtccccggggaagtga

SEQ ID NO: 32 - protein, 112 aa, Artificial Sequence
  Humanised Light Chain Variable Region L1
DVVMTQSPLSLPVTLGQPASISCRSSQSLENSNGKTYLNWFQQRPGQSPRRLIYGVSNRFSGVPDRFSGSGSGTDFTLKISRVEAEDVGVYFCLQVTHVPYTFGQGTKLEIK

SEQ ID NO: 33 - protein, 118 aa, Artificial Sequence
  Humanised Heavy Chain Variable Region H4
QVQLVQSGAEVKKPGSSVKVSCKASGYTFTNYWIGWVRQAPGQGLEWVGDIYPGGDYTNYNEKFKGRVTITADKSTSTAYMELSSLRSEDTAVYYCARWGLGYYFDYWGQGTMVTVSS

SEQ ID NO: 34 - protein, 112 aa, Artificial Sequence
  Humanised Light Chain Variable Region L2
DIVMTQTPLSLSVTPGQPASISCRSSQSLENSNGKTYLNWYLQKPGQSPQLLIYGVSNRFSGVPDRFSGSGSGTDFTLKISRVEAEDVGVYYCLQVTHVPYTFGQGTKVEIK

SEQ ID NO: 35 - protein, 118 aa, Artificial Sequence
  Humanised Heavy Chain Variable Region H2
QVQLVQSGPEVKKPGESLKISCKGSGYTFTNYWIGWVRQAPGKGLEWMGDIYPGGDYTNYNEKFKGQVTISADKSISTAYLQWSSLKASDTAIYYCARWGLGYYFDYWGRGTLVTVSS

SEQ ID NO: 36 - protein, 16 aa, Artificial Sequence
  VLCDR1 Variant 1
RSSQSLENSNAKTYLN

SEQ ID NO: 37 - protein, 16 aa, Artificial Sequence
  VLCDR1 Variant 2
RSSQSLENTNGKTYLN

SEQ ID NO: 38 - protein, 70 aa, Artificial Sequence
  Combined Sequence of CDRs of MDX-L1M2H4 & MDX-L2M2H2
RSSQSLENSNAKTYLNGVSNRFSLQVTHVPYTGYTFTNYWIGDIYPGGDYTNYNEKFKGARWGLGYYFDY

SEQ ID NO: 39 - protein, 70 aa, Artificial Sequence
  Combined Sequence of CDRs of MDX-L1M3H4 & MDX-L2M3H2
RSSQSLENTNGKTYLNGVSNRFSLQVTHVPYTGYTFTNYWIGDIYPGGDYTNYNEKFKGARWGLGYYFDY

SEQ ID NO: 40 - protein, 239 aa, Artificial Sequence
  MDX-L1H4 Light Chain
MVSSAQFLGLLLLCFQGTRCDVVMTQSPLSLPVTLGQPASISCRSSQSLENSNGKTYLNWFQQRPGQSPRRLIYGVSNRFSGVPDRFSGSGSGTDFTLKISRVEAEDVGVYFCLQVTHVPYTFGQGTKLEIKRTVAAPSVFIFPPSDEQLKSGTASVVCLLNNFYPREAKVQWKVDNALQSGNSQESVTEQDSKDSTYSLSSTLTLSKADYEKHKVYACEVTHQGLSSPVTKSFNRGEC

SEQ ID NO: 41 - protein, 467 aa, Artificial Sequence
  MDX-L1H4 Heavy Chain
MGWTLVFLFLLSVTAGVHSQVQLVQSGAEVKKPGSSVKVSCKASGYTFTNYWIGWVRQAPGQGLEWVGDIYPGGDYTNYNEKFKGRVTITADKSTSTAYMELSSLRSEDTAVYYCARWGLGYYFDYWGQGTMVTVSSASTKGPSVFPLAPSSKSTSGGTAALGCLVKDYFPEPVTVSWNSGALTSGVHTFPAVLQSSGLYSLSSVVTVPSSSLGTQTYICNVNHKPSNTKVDKKVEPKSCDKTHTCPPCPAPELLGGPSVFLFPPKPKDTLMISRTPEVTCVVVDVSHEDPEVKFNWYVDGVEVHNAKTKPREEQYNSTYRVVSVLTVLHQDWLNGKEYKCKVSNKALPAPIEKTISKAKGQPREPQVYTLPPSRDELTKNQVSLTCLVKGFYPSDIAVEWESNGQPENNYKTTPPVLDSDGSFFLYSKLTVDKSRWQQGNVFSCSVMHEALHNHYTQKSLSLSPGK

SEQ ID NO: 42 - protein, 239 aa, Artificial Sequence
  MDX-L2H2 Light Chain
MVSSAQFLGLLLLCFQGTRCDIVMTQTPLSLSVTPGQPASISCRSSQSLENSNGKTYLNWYLQKPGQSPQLLIYGVSNRFSGVPDRFSGSGSGTDFTLKISRVEAEDVGVYYCLQVTHVPYTFGQGTKVEIKRTVAAPSVFIFPPSDEQLKSGTASVVCLLNNFYPREAKVQWKVDNALQSGNSQESVTEQDSKDSTYSLSSTLTLSKADYEKHKVYACEVTHQGLSSPVTKSFNRGEC

SEQ ID NO: 43 - protein, 467 aa, Artificial Sequence
  MDX-L2H2 Heavy Chain
MGWTLVFLFLLSVTAGVHSQVQLVQSGPEVKKPGESLKISCKGSGYTFTNYWIGWVRQAPGKGLEWMGDIYPGGDYTNYNEKFKGQVTISADKSISTAYLQWSSLKASDTAIYYCARWGLGYYFDYWGRGTLVTVSSASTKGPSVFPLAPSSKSTSGGTAALGCLVKDYFPEPVTVSWNSGALTSGVHTFPAVLQSSGLYSLSSVVTVPSSSLGTQTYICNVNHKPSNTKVDKKVEPKSCDKTHTCPPCPAPELLGGPSVFLFPPKPKDTLMISRTPEVTCVVVDVSHEDPEVKFNWYVDGVEVHNAKTKPREEQYNSTYRVVSVLTVLHQDWLNGKEYKCKVSNKALPAPIEKTISKAKGQPREPQVYTLPPSRDELTKNQVSLTCLVKGFYPSDIAVEWESNGQPENNYKTTPPVLDSDGSFFLYSKLTVDKSRWQQGNVFSCSVMHEALHNHYTQKSLSLSPGK

SEQ ID NO: 44 - protein, 239 aa, Artificial Sequence
  MDX-L1M2H4 Light Chain
MVSSAQFLGLLLLCFQGTRCDVVMTQSPLSLPVTLGQPASISCRSSQSLENSNAKTYLNWFQQRPGQSPRRLIYGVSNRFSGVPDRFSGSGSGTDFTLKISRVEAEDVGVYFCLQVTHVPYTFGQGTKLEIKRTVAAPSVFIFPPSDEQLKSGTASVVCLLNNFYPREAKVQWKVDNALQSGNSQESVTEQDSKDSTYSLSSTLTLSKADYEKHKVYACEVTHQGLSSPVTKSFNRGEC

SEQ ID NO: 45 - protein, 239 aa, Artificial Sequence
  MDX-L2M2H2 Light Chain
MVSSAQFLGLLLLCFQGTRCDIVMTQTPLSLSVTPGQPASISCRSSQSLENSNAKTYLNWYLQKPGQSPQLLIYGVSNRFSGVPDRFSGSGSGTDFTLKISRVEAEDVGVYYCLQVTHVPYTFGQGTKVEIKRTVAAPSVFIFPPSDEQLKSGTASVVCLLNNFYPREAKVQWKVDNALQSGNSQESVTEQDSKDSTYSLSSTLTLSKADYEKHKVYACEVTHQGLSSPVTKSFNRGEC

SEQ ID NO: 46 - protein, 239 aa, Artificial Sequence
  MDX-L1M3H4 Light Chain
MVSSAQFLGLLLLCFQGTRCDVVMTQSPLSLPVTLGQPASISCRSSQSLENTNGKTYLNWFQQRPGQSPRRLIYGVSNRFSGVPDRFSGSGSGTDFTLKISRVEAEDVGVYFCLQVTHVPYTFGQGTKLEIKRTVAAPSVFIFPPSDEQLKSGTASVVCLLNNFYPREAKVQWKVDNALQSGNSQESVTEQDSKDSTYSLSSTLTLSKADYEKHKVYACEVTHQGLSSPVTKSFNRGEC

SEQ ID NO: 47 - protein, 239 aa, Artificial Sequence
  MDX-L2M3H2 Light Chain
MVSSAQFLGLLLLCFQGTRCDIVMTQTPLSLSVTPGQPASISCRSSQSLENTNGKTYLNWYLQKPGQSPQLLIYGVSNRFSGVPDRFSGSGSGTDFTLKISRVEAEDVGVYYCLQVTHVPYTFGQGTKVEIKRTVAAPSVFIFPPSDEQLKSGTASVVCLLNNFYPREAKVQWKVDNALQSGNSQESVTEQDSKDSTYSLSSTLTLSKADYEKHKVYACEVTHQGLSSPVTKSFNRGEC

SEQ ID NO: 48 - protein, 112 aa, Artificial Sequence
  MDX-L1M2H4 Light Chain Variable Region
DVVMTQSPLSLPVTLGQPASISCRSSQSLENSNAKTYLNWFQQRPGQSPRRLIYGVSNRFSGVPDRFSGSGSGTDFTLKISRVEAEDVGVYFCLQVTHVPYTFGQGTKLEIK

SEQ ID NO: 49 - protein, 112 aa, Artificial Sequence
  MDX-L1M3H4 Light Chain Variable Region
DVVMTQSPLSLPVTLGQPASISCRSSQSLENTNGKTYLNWFQQRPGQSPRRLIYGVSNRFSGVPDRFSGSGSGTDFTLKISRVEAEDVGVYFCLQVTHVPYTFGQGTKLEIK

SEQ ID NO: 50 - protein, 112 aa, Artificial Sequence
  MDX-L2M2H2 Light Chain Variable Region
DIVMTQTPLSLSVTPGQPASISCRSSQSLENSNAKTYLNWYLQKPGQSPQLLIYGVSNRFSGVPDRFSGSGSGTDFTLKISRVEAEDVGVYYCLQVTHVPYTFGQGTKVEIK

SEQ ID NO: 51 - protein, 112 aa, Artificial Sequence
  MDX-L2M3H2 Light Chain Variable Region
DIVMTQTPLSLSVTPGQPASISCRSSQSLENTNGKTYLNWYLQKPGQSPQLLIYGVSNRFSGVPDRFSGSGSGTDFTLKISRVEAEDVGVYYCLQVTHVPYTFGQGTKVEIK

SEQ ID NO: 52 - protein, 20 aa, Artificial Sequence
  Signal Sequence of Humanised Light Chains
MVSSAQFLGLLLLCFQGTRC

SEQ ID NO: 53 - protein, 19 aa, Artificial Sequence
  Signal Sequence of Humanised Heavy Chains
MGWTLVFLFLLSVTAGVHS

SEQ ID NO: 54 - protein, 219 aa, Artificial Sequence
  MDX-L1M2H4 Mature Light Chain
DVVMTQSPLSLPVTLGQPASISCRSSQSLENSNAKTYLNWFQQRPGQSPRRLIYGVSNRFSGVPDRFSGSGSGTDFTLKISRVEAEDVGVYFCLQVTHVPYTFGQGTKLEIKRTVAAPSVFIFPPSDEQLKSGTASVVCLLNNFYPREAKVQWKVDNALQSGNSQESVTEQDSKDSTYSLSSTLTLSKADYEKHKVYACEVTHQGLSSPVTKSFNRGEC

SEQ ID NO: 55 - protein, 448 aa, Artificial Sequence
  MDX-L1H4 Mature Heavy Chain
QVQLVQSGAEVKKPGSSVKVSCKASGYTFTNYWIGWVRQAPGQGLEWVGDIYPGGDYTNYNEKFKGRVTITADKSTSTAYMELSSLRSEDTAVYYCARWGLGYYFDYWGQGTMVTVSSASTKGPSVFPLAPSSKSTSGGTAALGCLVKDYFPEPVTVSWNSGALTSGVHTFPAVLQSSGLYSLSSVVTVPSSSLGTQTYICNVNHKPSNTKVDKKVEPKSCDKTHTCPPCPAPELLGGPSVFLFPPKPKDTLMISRTPEVTCVVVDVSHEDPEVKFNWYVDGVEVHNAKTKPREEQYNSTYRVVSVLTVLHQDWLNGKEYKCKVSNKALPAPIEKTISKAKGQPREPQVYTLPPSRDELTKNQVSLTCLVKGFYPSDIAVEWESNGQPENNYKTTPPVLDSDGSFFLYSKLTVDKSRWQQGNVFSCSVMHEALHNHYTQKSLSLSPGK

SEQ ID NO: 56 - protein, 16 aa, Artificial Sequence
  VLCDR1 "mod1"
RSSQSLENSDGKTYLN

SEQ ID NO: 57 - DNA, 720 bp, Artificial Sequence
  MDX-L1M2H4 Light Chain
atggtgtcatccgctcaatttctcggtttgcttctcctgtgtttccaaggcacccgctgcgacgtggtcatgacccagagcccactgagccttccggtcaccttgggacagcccgcctcaatttcatgccggtccagccagtccctggagaactccaacgccaagacctatctgaactggttccagcagcgccctggacagtccccgaggcgcctgatctacggcgtcagcaacaggttctcgggcgtgccggacagattctccggctccggaagcggaactgacttcaccctgaaaatctcaagagtggaagccgaggacgtgggcgtgtacttctgcctccaagtcacgcacgtgccgtacactttcggacaagggactaagctggagatcaagcggaccgtggcggccccctctgtgttcattttccctccctcggacgaacagctgaagtcgggaacagcctccgtcgtgtgcctgctcaacaacttctacccccgggaagcgaaggtccagtggaaagtggataacgcactccaatcggggaactcccaggaatccgtgactgagcaggactcgaaggattccacttactccctgtcgtccaccctgactctgagcaaggccgactacgagaagcataaggtctacgcctgcgaagtgacccaccagggtctgagctcccctgtgaccaagagctttaatcggggcgaatgttga

SEQ ID NO: 58 - DNA, 1404 bp, Artificial Sequence
  MDX-L1H4 Heavy Chain
atgggatggactctcgtgttcctttttctcctctctgtcactgccggggtgcattcgcaagtccagctggtgcagtcgggagcagaggtgaaaaagcccggatcgtcagtgaaggtcagctgcaaagcctcgggatacactttcaccaactactggattggatgggtcagacaggcccccggccaaggactggagtgggtcggcgacatctaccctgggggcgactataccaactacaacgaaaagttcaagggacgcgtgacaattaccgccgataagagcaccagcactgcctacatggagcttagctcattgcggtccgaggataccgctgtgtactactgtgcgcggtggggccttggttactacttcgactactggggacagggtaccatggtcacggtgtcctccgcgtccaccaagggtccctccgtgttccctctcgcgccgtcctcaaagtctacctccggtggaactgccgcgctcggttgtctcgtgaaggactacttcccggagcctgtgactgtctcctggaactccggggccctcaccagcggagtgcacactttccccgccgtgctgcaatcctccggcctgtacagcctgtcctccgtcgtgactgtgcctagctcctccctgggaacccagacctacatctgcaacgtgaaccacaagccctccaacaccaaggtcgacaagaaggtcgaaccgaagtcgtgcgacaagactcatacgtgccctccttgcccggccccggaactgctgggaggcccatccgtgttcctgttcccacccaagcctaaggataccctgatgatcagcagaacaccggaagtgacctgtgtggtggtggacgtcagccacgaagatcccgaggtcaagttcaattggtacgtggacggggtggaggtgcacaacgcaaagaccaagccccgggaggaacagtacaactccacctatcgcgtggtgtcggtgctgacggtgctgcaccaggactggttgaacggaaaggagtataagtgcaaagtgtcgaacaaggccctgcccgctcctatcgaaaagaccatctccaaggccaagggccagccgcgggaaccccaggtctacactctcccaccgagccgcgacgaactgactaagaatcaagtgtcgctgacttgcctcgtcaagggcttctacccgtccgacatcgccgtggaatgggagagcaacggccagccggaaaacaactacaagaccacccctcccgtgctggattccgacgggtccttcttcctgtactcaaaactgaccgtggataagtccagatggcagcagggcaatgtcttttcatgctccgtgatgcacgaggctctgcataaccactacacccagaagtcgctgtccctgtccccggggaagtga

SEQ ID NO: 59 - DNA, 336 bp, Artificial Sequence
  MDX-L1M2H4 Light Chain Variable Region
gacgtggtcatgacccagagcccactgagccttccggtcaccttgggacagcccgcctcaatttcatgccggtccagccagtccctggagaactccaacgccaagacctatctgaactggttccagcagcgccctggacagtccccgaggcgcctgatctacggcgtcagcaacaggttctcgggcgtgccggacagattctccggctccggaagcggaactgacttcaccctgaaaatctcaagagtggaagccgaggacgtgggcgtgtacttctgcctccaagtcacgcacgtgccgtacactttcggacaagggactaagctggagatcaag

SEQ ID NO: 60 - DNA, 354 bp, Artificial Sequence
  MDX-L1H4 Heavy Chain Variable Region
caagtccagctggtgcagtcgggagcagaggtgaaaaagcccggatcgtcagtgaaggtcagctgcaaagcctcgggatacactttcaccaactactggattggatgggtcagacaggcccccggccaaggactggagtgggtcggcgacatctaccctgggggcgactataccaactacaacgaaaagttcaagggacgcgtgacaattaccgccgataagagcaccagcactgcctacatggagcttagctcattgcggtccgaggataccgctgtgtactactgtgcgcggtggggccttggttactacttcgactactggggacagggtaccatggtcacggtgtcctcc

SEQ ID NO: 61 - DNA, 720 bp, Artificial Sequence
  MDX-L2M2H2 Ligh Chain
atggtgtcatccgctcaatttctcggtttgcttctcctgtgtttccaaggcacccgctgcgacatcgtcatgacccagaccccattgagcctttccgtcacgccgggacagcccgcctccatttcctgccgctcaagccagtccctggagaactcaaacgccaagacctacctgaattggtatctgcagaagcctggacagagcccgcagctgctgatctacggcgtcagcaacaggttctcgggcgtgccggacagattctccggctccggaagcggaactgacttcaccctgaaaatctcacgcgtggaagccgaggacgtgggcgtgtactactgcctccaagtcacccacgtgccgtacactttcggacaagggactaaggtcgagatcaagcggaccgtggcggccccctctgtgttcattttccctccctcggacgaacagctgaagtcgggaacagcctccgtcgtgtgcctgctcaacaacttctacccccgggaagcgaaggtccagtggaaagtggataacgcactccaatcggggaactcccaggaatccgtgactgagcaggactcgaaggattccacttactccctgtcgtccaccctgactctgagcaaggccgactacgagaagcataaggtctacgcctgcgaagtgacccaccagggtctgagctcccctgtgaccaagagctttaatcggggcgaatgttga

SEQ ID NO: 62 - DNA, 1404 bp, Artificial Sequence
  MDX-L2H2 Heavy Chain
atgggatggactctcgtgttcctttttctcctctctgtcactgccggggtgcattcgcaagtccagctggtgcagtcgggaccagaggtgaaaaagcccggagagtcacttaagatcagctgcaaaggctcgggatacactttcaccaactactggattggttgggtcagacaggcccccggcaaaggactggagtggatgggcgacatctaccctgggggcgactataccaactacaacgaaaagttcaagggacaagtgacaatttcggccgataagagcattagcactgcataccttcagtggagctcattgaaggcctccgataccgctatctactactgtgcgcggtggggcctgggatactacttcgactactggggaaggggtaccttggtcacggtgtcctccgcgtccaccaagggtccctccgtgttccctctcgcgccgtcctcaaagtctacctccggtggaactgccgcgctcggttgtctcgtgaaggactacttcccggagcctgtgactgtctcctggaactccggggccctcaccagcggagtgcacactttccccgccgtgctgcaatcctccggcctgtacagcctgtcctccgtcgtgactgtgcctagctcctccctgggaacccagacctacatctgcaacgtgaaccacaagccctccaacaccaaggtcgacaagaaggtcgaaccgaagtcgtgcgacaagactcatacgtgccctccttgcccggccccggaactgctgggaggcccatccgtgttcctgttcccacccaagcctaaggataccctgatgatcagcagaacaccggaagtgacctgtgtggtggtggacgtcagccacgaagatcccgaggtcaagttcaattggtacgtggacggggtggaggtgcacaacgcaaagaccaagccccgggaggaacagtacaactccacctatcgcgtggtgtcggtgctgacggtgctgcaccaggactggttgaacggaaaggagtataagtgcaaagtgtcgaacaaggccctgcccgctcctatcgaaaagaccatctccaaggccaagggccagccgcgggaaccccaggtctacactctcccaccgagccgcgacgaactgactaagaatcaagtgtcgctgacttgcctcgtcaagggcttctacccgtccgacatcgccgtggaatgggagagcaacggccagccggaaaacaactacaagaccacccctcccgtgctggattccgacgggtccttcttcctgtactcaaaactgaccgtggataagtccagatggcagcagggcaatgtcttttcatgctccgtgatgcacgaggctctgcataaccactacacccagaagtcgctgtccctgtccccggggaagtga

SEQ ID NO: 63 - DNA, 336 bp, Artificial Sequence
  MDX-L2M2H2 Light Chain Variable Region
gacatcgtcatgacccagaccccattgagcctttccgtcacgccgggacagcccgcctccatttcctgccgctcaagccagtccctggagaactcaaacgccaagacctacctgaattggtatctgcagaagcctggacagagcccgcagctgctgatctacggcgtcagcaacaggttctcgggcgtgccggacagattctccggctccggaagcggaactgacttcaccctgaaaatctcacgcgtggaagccgaggacgtgggcgtgtactactgcctccaagtcacccacgtgccgtacactttcggacaagggactaaggtcgagatcaag

SEQ ID NO: 64 - DNA, 354 bp, Artificial Sequence
  MDX-L2H2 Heavy Chain Variable Region
caagtccagctggtgcagtcgggaccagaggtgaaaaagcccggagagtcacttaagatcagctgcaaaggctcgggatacactttcaccaactactggattggttgggtcagacaggcccccggcaaaggactggagtggatgggcgacatctaccctgggggcgactataccaactacaacgaaaagttcaagggacaagtgacaatttcggccgataagagcattagcactgcataccttcagtggagctcattgaaggcctccgataccgctatctactactgtgcgcggtggggcctgggatactacttcgactactggggaaggggtaccttggtcacggtgtcctcc

SEQ ID NO: 65 - DNA, 48 bp, Artificial Sequence
  MDX-L1M2H4 VLCDR1
cggtccagccagtccctggagaactccaacgccaagacctatctgaac

SEQ ID NO: 66 - DNA, 48 bp, Artificial Sequence
  MDX-L2M2H2 VLCDR1
cgctcaagccagtccctggagaactcaaacgccaagacctacctgaat

SEQ ID NO: 67 - DNA, 21 bp, Artificial Sequence
  MDX-L1H4 & MDX-L2H2 VLCDR2
ggcgtcagcaacaggttctcg

SEQ ID NO: 68 - DNA, 27 bp, Artificial Sequence
  MDX-L1H4 VLCDR3
ctccaagtcacgcacgtgccgtacact

SEQ ID NO: 69 - DNA, 27 bp, Artificial Sequence
  MDX-L2H2 VLCDR3
ctccaagtcacccacgtgccgtacact

SEQ ID NO: 70 - DNA, 30 bp, Artificial Sequence
  MDX-L1H4 VHCDR1
ggatacactttcaccaactactggattgga

SEQ ID NO: 71 - DNA, 30 bp, Artificial Sequence
  MDX-L2H2 VHCDR1
ggatacactttcaccaactactggattggt

SEQ ID NO: 72 - DNA, 51 bp, Artificial Sequence
  MDX-L1H4 & MDX-L2H2 VHCDR2
gacatctaccctgggggcgactataccaactacaacgaaaagttcaaggga

SEQ ID NO: 73 - DNA, 33 bp, Artificial Sequence
  MDX-L1H4 VHCDR3
gcgcggtggggccttggttactacttcgactac

SEQ ID NO: 74 - DNA, 33 bp, Artificial Sequence
  MDX-L2H2 VHCDR3
gcgcggtggggcctgggatactacttcgactac

SEQ ID NO: 75 - protein, 219 aa, Artificial Sequence
  MDX-L1H4 Mature Light Chain
DVVMTQSPLSLPVTLGQPASISCRSSQSLENSNGKTYLNWFQQRPGQSPRRLIYGVSNRFSGVPDRFSGSGSGTDFTLKISRVEAEDVGVYFCLQVTHVPYTFGQGTKLEIKRTVAAPSVFIFPPSDEQLKSGTASVVCLLNNFYPREAKVQWKVDNALQSGNSQESVTEQDSKDSTYSLSSTLTLSKADYEKHKVYACEVTHQGLSSPVTKSFNRGEC

SEQ ID NO: 76 - protein, 219 aa, Artificial Sequence
  MDX-L1M3H4 Mature Light Chain
DVVMTQSPLSLPVTLGQPASISCRSSQSLENTNGKTYLNWFQQRPGQSPRRLIYGVSNRFSGVPDRFSGSGSGTDFTLKISRVEAEDVGVYFCLQVTHVPYTFGQGTKLEIKRTVAAPSVFIFPPSDEQLKSGTASVVCLLNNFYPREAKVQWKVDNALQSGNSQESVTEQDSKDSTYSLSSTLTLSKADYEKHKVYACEVTHQGLSSPVTKSFNRGEC

SEQ ID NO: 77 - protein, 219 aa, Artificial Sequence
  MDX-L2H2 Mature Light Chain
DIVMTQTPLSLSVTPGQPASISCRSSQSLENSNGKTYLNWYLQKPGQSPQLLIYGVSNRFSGVPDRFSGSGSGTDFTLKISRVEAEDVGVYYCLQVTHVPYTFGQGTKVEIKRTVAAPSVFIFPPSDEQLKSGTASVVCLLNNFYPREAKVQWKVDNALQSGNSQESVTEQDSKDSTYSLSSTLTLSKADYEKHKVYACEVTHQGLSSPVTKSFNRGEC

SEQ ID NO: 78 - protein, 219 aa, Artificial Sequence
  MDX-L2M2H2 Mature Light Chain
DIVMTQTPLSLSVTPGQPASISCRSSQSLENSNAKTYLNWYLQKPGQSPQLLIYGVSNRFSGVPDRFSGSGSGTDFTLKISRVEAEDVGVYYCLQVTHVPYTFGQGTKVEIKRTVAAPSVFIFPPSDEQLKSGTASVVCLLNNFYPREAKVQWKVDNALQSGNSQESVTEQDSKDSTYSLSSTLTLSKADYEKHKVYACEVTHQGLSSPVTKSFNRGEC

SEQ ID NO: 79 - protein, 219 aa, Artificial Sequence
  MDX-L2M3H2 Mature Light Chain
DIVMTQTPLSLSVTPGQPASISCRSSQSLENTNGKTYLNWYLQKPGQSPQLLIYGVSNRFSGVPDRFSGSGSGTDFTLKISRVEAEDVGVYYCLQVTHVPYTFGQGTKVEIKRTVAAPSVFIFPPSDEQLKSGTASVVCLLNNFYPREAKVQWKVDNALQSGNSQESVTEQDSKDSTYSLSSTLTLSKADYEKHKVYACEVTHQGLSSPVTKSFNRGEC

SEQ ID NO: 80 - protein, 448 aa, Artificial Sequence
  MDX-L2H2 Mature Heavy Chain
QVQLVQSGPEVKKPGESLKISCKGSGYTFTNYWIGWVRQAPGKGLEWMGDIYPGGDYTNYNEKFKGQVTISADKSISTAYLQWSSLKASDTAIYYCARWGLGYYFDYWGRGTLVTVSSASTKGPSVFPLAPSSKSTSGGTAALGCLVKDYFPEPVTVSWNSGALTSGVHTFPAVLQSSGLYSLSSVVTVPSSSLGTQTYICNVNHKPSNTKVDKKVEPKSCDKTHTCPPCPAPELLGGPSVFLFPPKPKDTLMISRTPEVTCVVVDVSHEDPEVKFNWYVDGVEVHNAKTKPREEQYNSTYRVVSVLTVLHQDWLNGKEYKCKVSNKALPAPIEKTISKAKGQPREPQVYTLPPSRDELTKNQVSLTCLVKGFYPSDIAVEWESNGQPENNYKTTPPVLDSDGSFFLYSKLTVDKSRWQQGNVFSCSVMHEALHNHYTQKSLSLSPGK

SEQ ID NO: 81 - DNA, 720 bp, Artificial Sequence
  MDX-L1H4 Light Chain
atggtgtcatccgctcaatttctcggtttgcttctcctgtgtttccaaggcacccgctgcgacgtggtcatgacccagagcccactgagccttccggtcaccttgggacagcccgcctcaatttcatgccggtccagccagtccctggagaactccaacggaaagacctatctgaactggttccagcagcgccctggacagtccccgaggcgcctgatctacggcgtcagcaacaggttctcgggcgtgccggacagattctccggctccggaagcggaactgacttcaccctgaaaatctcaagagtggaagccgaggacgtgggcgtgtactactgcctccaagtcacgcacgtgccgtacactttcggacaagggactaagctggagatcaagcggaccgtggcggccccctctgtgttcattttccctccctcggacgaacagctgaagtcgggaacagcctccgtcgtgtgcctgctcaacaacttctacccccgggaagcgaaggtccagtggaaagtggataacgcactccaatcggggaactcccaggaatccgtgactgagcaggactcgaaggattccacttactccctgtcgtccaccctgactctgagcaaggccgactacgagaagcataaggtctacgcctgcgaagtgacccaccagggtctgagctcccctgtgaccaagagctttaatcggggcgaatgttga

SEQ ID NO: 82 - DNA, 336 bp, Artificial Sequence
  MDX-L1H4 Light Chain Variable Region
gacgtggtcatgacccagagcccactgagccttccggtcaccttgggacagcccgcctcaatttcatgccggtccagccagtccctggagaactccaacggaaagacctatctgaactggttccagcagcgccctggacagtccccgaggcgcctgatctacggcgtcagcaacaggttctcgggcgtgccggacagattctccggctccggaagcggaactgacttcaccctgaaaatctcaagagtggaagccgaggacgtgggcgtgtactactgcctccaagtcacgcacgtgccgtacactttcggacaagggactaagctggagatcaag

SEQ ID NO: 83 - DNA, 720 bp, Artificial Sequence
  MDX-L2H2 Light Chain
atggtgtcatccgctcaatttctcggtttgcttctcctgtgtttccaaggcacccgctgcgacatcgtcatgacccagaccccattgagcctttccgtcacgccgggacagcccgcctccatttcctgccgctcaagccagtccctggagaactcaaacggaaagacctacctgaattggtatctgcagaagcctggacagagcccgcagctgctgatctacggcgtcagcaacaggttctcgggcgtgccggacagattctccggctccggaagcggaactgacttcaccctgaaaatctcacgcgtggaagccgaggacgtgggcgtgtactactgcctccaagtcacccacgtgccgtacactttcggacaagggactaaggtcgagatcaagcggaccgtggcggccccctctgtgttcattttccctccctcggacgaacagctgaagtcgggaacagcctccgtcgtgtgcctgctcaacaacttctacccccgggaagcgaaggtccagtggaaagtggataacgcactccaatcggggaactcccaggaatccgtgactgagcaggactcgaaggattccacttactccctgtcgtccaccctgactctgagcaaggccgactacgagaagcataaggtctacgcctgcgaagtgacccaccagggtctgagctcccctgtgaccaagagctttaatcggggcgaatgttga

SEQ ID NO: 84 - DNA, 336 bp, Artificial Sequence
  MDX-L2H2 Ligh Chain Variable Region
gacatcgtcatgacccagaccccattgagcctttccgtcacgccgggacagcccgcctccatttcctgccgctcaagccagtccctggagaactcaaacggaaagacctacctgaattggtatctgcagaagcctggacagagcccgcagctgctgatctacggcgtcagcaacaggttctcgggcgtgccggacagattctccggctccggaagcggaactgacttcaccctgaaaatctcacgcgtggaagccgaggacgtgggcgtgtactactgcctccaagtcacccacgtgccgtacactttcggacaagggactaaggtcgagatcaag

SEQ ID NO: 85 - DNA, 48 bp, Artificial Sequence
  MDX-L1H4 VLCDR1
cggtccagccagtccctggagaactccaacggaaagacctatctgaac

SEQ ID NO: 86 - DNA, 48 bp, Artificial Sequence
  MDX-L2H2 VLCDR1
cgctcaagccagtccctggagaactcaaacggaaagacctacctgaat

SEQ ID NO: 87 - DNA, 48 bp, Artificial Sequence
  MDX-L1M3H4 VLCDR1
cggtccagccagtccctggagaacaccaacggaaagacctatctgaac

SEQ ID NO: 88 - DNA, 48 bp, Artificial Sequence
  MDX-L2M3H2 VLCDR1
cgctcaagccagtccctggagaacaccaacggaaagacctacctgaat

SEQ ID NO: 89 - DNA, 720 bp, Artificial Sequence
  MDX-L1M3H4 Light Chain
atggtgtcatccgctcaatttctcggtttgcttctcctgtgtttccaaggcacccgctgcgacgtggtcatgacccagagcccactgagccttccggtcaccttgggacagcccgcctcaatttcatgccggtccagccagtccctggagaacaccaacggaaagacctatctgaactggttccagcagcgccctggacagtccccgaggcgcctgatctacggcgtcagcaacaggttctcgggcgtgccggacagattctccggctccggaagcggaactgacttcaccctgaaaatctcaagagtggaagccgaggacgtgggcgtgtacttctgcctccaagtcacgcacgtgccgtacactttcggacaagggactaagctggagatcaagcggaccgtggcggccccctctgtgttcattttccctccctcggacgaacagctgaagtcgggaacagcctccgtcgtgtgcctgctcaacaacttctacccccgggaagcgaaggtccagtggaaagtggataacgcactccaatcggggaactcccaggaatccgtgactgagcaggactcgaaggattccacttactccctgtcgtccaccctgactctgagcaaggccgactacgagaagcataaggtctacgcctgcgaagtgacccaccagggtctgagctcccctgtgaccaagagctttaatcggggcgaatgttga

SEQ ID NO: 90 - DNA, 336 bp, Artificial Sequence
  MDX-L1M3H4 Light Chain Variable Region
gacgtggtcatgacccagagcccactgagccttccggtcaccttgggacagcccgcctcaatttcatgccggtccagccagtccctggagaacaccaacggaaagacctatctgaactggttccagcagcgccctggacagtccccgaggcgcctgatctacggcgtcagcaacaggttctcgggcgtgccggacagattctccggctccggaagcggaactgacttcaccctgaaaatctcaagagtggaagccgaggacgtgggcgtgtacttctgcctccaagtcacgcacgtgccgtacactttcggacaagggactaagctggagatcaag

SEQ ID NO: 91 - DNA, 720 bp, Artificial Sequence
  MDX-L2M3H2 Light Chain
atggtgtcatccgctcaatttctcggtttgcttctcctgtgtttccaaggcacccgctgcgacatcgtcatgacccagaccccattgagcctttccgtcacgccgggacagcccgcctccatttcctgccgctcaagccagtccctggagaacaccaacggaaagacctacctgaattggtatctgcagaagcctggacagagcccgcagctgctgatctacggcgtcagcaacaggttctcgggcgtgccggacagattctccggctccggaagcggaactgacttcaccctgaaaatctcacgcgtggaagccgaggacgtgggcgtgtactactgcctccaagtcacccacgtgccgtacactttcggacaagggactaaggtcgagatcaagcggaccgtggcggccccctctgtgttcattttccctccctcggacgaacagctgaagtcgggaacagcctccgtcgtgtgcctgctcaacaacttctacccccgggaagcgaaggtccagtggaaagtggataacgcactccaatcggggaactcccaggaatccgtgactgagcaggactcgaaggattccacttactccctgtcgtccaccctgactctgagcaaggccgactacgagaagcataaggtctacgcctgcgaagtgacccaccagggtctgagctcccctgtgaccaagagctttaatcggggcgaatgttga

SEQ ID NO: 92 - DNA, 336 bp, Artificial Sequence
  MDX-L2M3H2 Light Chain Variable Region
gacatcgtcatgacccagaccccattgagcctttccgtcacgccgggacagcccgcctccatttcctgccgctcaagccagtccctggagaacaccaacggaaagacctacctgaattggtatctgcagaagcctggacagagcccgcagctgctgatctacggcgtcagcaacaggttctcgggcgtgccggacagattctccggctccggaagcggaactgacttcaccctgaaaatctcacgcgtggaagccgaggacgtgggcgtgtactactgcctccaagtcacccacgtgccgtacactttcggacaagggactaaggtcgagatcaag